European Patent Application EP 4 595 974 A2, published August 6, 2025. Title: THERAPEUTIC COMBINATIONS OF TDFRPS AND ADDITIONAL AGENTS AND METHODS OF USE. Applicant: William Dean Carlson. Application EP 25161427.7, filed March 3, 2025. The sequence listing filed with the application follows.

SEQUENCE LISTING (4 sequences)

SEQ ID NO: 1 - protein, 16 aa, synthetic construct
  REGION 1..16: note = Description of Artificial Sequence: Synthetic peptide
CYFDDSSNVLCKKYRS

SEQ ID NO: 2 - protein, 16 aa, synthetic construct
  REGION 1..16: note = Description of Artificial Sequence: Synthetic peptide
CYFDDSSQVICKKYRS

SEQ ID NO: 3 - protein, 16 aa, synthetic construct
  REGION 1..16: note = Description of Artificial Sequence: Synthetic peptide
CYYDNSSSVLCKRYRS

SEQ ID NO: 4 - protein, 16 aa, synthetic construct
  REGION 1..16: note = Description of Artificial Sequence: Synthetic peptide
  MOD_RES 14: note = D-Tyr
CYYDNSSSVLCKRYRS